European Patent Application EP 4 349 868 A2, published April 10, 2024. Title: Humanized and Chimeric Monoclonal Antibodies to CD47. Applicant: The Board of Trustees of the Leland Stanford Junior University. The sequence listing filed with the application follows.

SEQUENCE LISTING (48 sequences)

SEQ ID NO: 1 - protein, 118 aa, Mus musculus
EVQLVESGGDLVKPGGSLKLSCAASGFTFSGYGMSWVRQTPDKRLEWVATITSGGTYTYYPDSVKGRFTISRDNAKNTLYLQIDSLKSEDTAIYFCARSLAGNAMDYWGQGTSVTVSS

SEQ ID NO: 2 - protein, 107 aa, Mus musculus
DIVMTQSPATLSVTPGDRVSLSCRASQTISDYLHWYQQKSHESPRLLIKFASQSISGIPSRFSGSGSGSDFTLSINSVEPEDVGVYYCQNGHGFPRTFGGGTKLEIK

SEQ ID NO: 3 - protein, 5 aa, synthetic construct
  REGION 1..5: note = B6H12 heavy chain CDR1
GYGMS

SEQ ID NO: 4 - protein, 17 aa, synthetic construct
  REGION 1..17: note = B6H12 heavy chain CDR2
TITSGGTYTYYPDSVKG

SEQ ID NO: 5 - protein, 9 aa, synthetic construct
  REGION 1..9: note = B6H12 heavy chain CDR3
SLAGNAMDY

SEQ ID NO: 6 - protein, 11 aa, synthetic construct
  REGION 1..11: note = B6H12 light chain CDR1
RASQTISDYLH

SEQ ID NO: 7 - protein, 7 aa, synthetic construct
  REGION 1..7: note = B6H12 light chain CDR2
FASQSIS

SEQ ID NO: 8 - protein, 9 aa, synthetic construct
  REGION 1..9: note = B6H12 light chain CDR3
QNGHGFPRT

SEQ ID NO: 9 - DNA, 354 bp, synthetic construct
  misc_feature 1..354: note = Humanized B6H12 heavy chain
  source 1..354: mol_type = other DNA
gaggtgcagctggtggagtctgggggaggcttggtccagcctggggggtccctgagactctcctgtgcagcctctggattcacctttagtggctatggcatgagctgggtccgccaggctccagggaaggggctggagtgggtggccaccataactagtggtggaacttacacctactatccagactctgtgaagggccgattcaccatctccagagacaacgccaagaactcactgtatctgcaaatgaacagcctgagagccgaggacacggctgtgtattactgtgcgagatccctcgcgggaaatgctatggactactggggccaaggaaccctggtcaccgtctcctca

SEQ ID NO: 10 - DNA, 321 bp, synthetic construct
  misc_feature 1..321: note = Humanized B6H12 light chain
  source 1..321: mol_type = other DNA
gaaattgtgttgacacagtctccagccaccctgtctttgtctccaggggaaagagccaccctctcctgcagggccagtcagactattagcgactacttacactggtaccaacagaaacctggccaggctcccaggctcctcatcaaatttgcatcccaatccatttctggcatcccagccaggttcagtggcagtgggtctgggacagacttcactctcaccatcagcagcctagagcctgaagattttgcagtttattactgtcagaatggtcacggctttcctcggacgttcggccaagggaccaaggtggaaatcaaa

SEQ ID NO: 11 - protein, 118 aa, synthetic construct
  REGION 1..118: note = Humanized B6H12 VH
EVQLVESGGGLVQPGGSLRLSCAASGFTFSGYGMSWVRQAPGKGLEWVATITSGGTYTYYPDSVKGRFTISRDNAKNSLYLQMNSLRAEDTAVYYCARSLAGNAMDYWGQGTLVTVSS

SEQ ID NO: 12 - protein, 107 aa, synthetic construct
  REGION 1..107: note = Humanized B6H12 VL
EIVLTQSPATLSLSPGERATLSCRASQTISDYLHWYQQKPGQAPRLLIKFASQSISGIPARFSGSGSGTDFTLTISSLEPEDFAVYYCQNGHGFPRTFGQGTKVEIK

SEQ ID NO: 13 - DNA, 411 bp, Mus musculus
  source 1..411: mol_type = unassigned DNA
atgaacttcgggctcagcttgattttccttgccctcattttaaaaggtgtccagtgtgaggtgcagctggtggagtctgggggagacttagtgaagcctggagggtccctgaaactctcctgtgcagcctctggattcactttcagtggctatggcatgtcttgggttcgccagactccagacaagaggctggagtgggtcgcaaccattactagtggtggtacttacacctactatccagacagtgtgaaggggcgattcaccatctccagagacaatgccaagaacaccctgtacctgcaaatagacagtctgaagtctgaggatacagccatatatttctgtgcaagatccctcgcgggaaatgctatggactactggggtcaaggaacctcagtcaccgtctcctca

SEQ ID NO: 14 - DNA, 381 bp, Mus musculus
  source 1..381: mol_type = unassigned DNA
atggtgtccacttctcagctccttggacttttgcttttctggacttcagcctccagatgtgacattgtgatgactcagtctccagccaccctgtctgtgactccaggagatagagtctctctttcctgcagggccagccagactattagcgactacttacactggtatcaacaaaaatcacatgagtctccaaggcttctcatcaaatttgcttcccaatccatttctgggatcccctccaggttcagtggcagtggatcaggctcagatttcactctcagtatcaacagtgtggaacctgaagatgttggagtgtattactgtcaaaatggtcacggctttcctcggacgttcggtggaggcaccaagctggaaatcaaa

SEQ ID NO: 15-16 - skipped (2 entries)

SEQ ID NO: 17 - protein, 118 aa, synthetic construct
  REGION 1..118: note = Humanized B6H12 VH
EVQLLESGGGLVQPGGSLRLSCAASGFTFSGYGMSWVRQAPGKGLEWVATITSGGTYTYYPDSVKGRFTISRDNSKNTLYLQMNSLRAEDTAVYYCARSLAGNAMDYWGQGTLVTVSS

SEQ ID NO: 18 - protein, 117 aa, synthetic construct
  REGION 1..117: note = 5F9 heavy chain variable region
QVQLQQPGAELVKPGASVMMSCKASGYTFTNYNMHWVKQTPGQGLEWIGTIYPGNDDTSYNQKFKDKATLTADKSSSAAYMQLSSLTSEDSAVYYCARGGYRAMDYWGQGTSVTVSS

SEQ ID NO: 19 - protein, 112 aa, synthetic construct
  REGION 1..112: note = 5F9 light chain variable region
DVLMTQTPLSLPVSLGDQASISCRSSQSIVYSNGNTYLGWYLQKPGQSPKLLIYKVSNRFSGVPDRFSGSGSGTDFTLKISRVEAEDLGVYHCFQGSHVPYTFGGGTKVEIK

SEQ ID NO: 20 - protein, 5 aa, synthetic construct
  REGION 1..5: note = 5F9 heavy chain CDR1
NYNMH

SEQ ID NO: 21 - protein, 17 aa, synthetic construct
  REGION 1..17: note = 5F9 heavy chain CDR2
TIYPGNDDTSYNQKFKD

SEQ ID NO: 22 - protein, 8 aa, synthetic construct
  REGION 1..8: note = 5F9 heavy chain CDR3
GGYRAMDY

SEQ ID NO: 23 - protein, 16 aa, synthetic construct
  REGION 1..16: note = 5F9 light chain CDR1
RSSQSIVYSNGNTYLG

SEQ ID NO: 24 - protein, 7 aa, synthetic construct
  REGION 1..7: note = 5F9 light chain CDR2
KVSNRFS

SEQ ID NO: 25 - protein, 9 aa, synthetic construct
  REGION 1..9: note = 5F9 light chain CDR3
FQGSHVPYT

SEQ ID NO: 26 - protein, 120 aa, Mus musculus
EVQLQQSGPELVKPGASVKMSCKASGYTFTTYVVHWVKQTPGQGLEWIGYINPYNDGTKYNEKFKGKATLTSDKSSSTAYMEFSSLTSEDSAVYYCVRGYYRYGYTMDYWGQGTSVTVSS

SEQ ID NO: 27 - protein, 107 aa, Mus musculus
DIVMTQSPATLSVTPGDRVSLSCRASQNFSDYLHWYQQKSHESPRLLIKYVSHSISGIPSRFSGSGSGSDFTLSINSVEPEDVGVYYCQNGHSFPPTFGGGTKLEIK

SEQ ID NO: 28 - protein, 5 aa, synthetic construct
  REGION 1..5: note = 8B6 heavy chain CDR1
TYVVH

SEQ ID NO: 29 - protein, 17 aa, synthetic construct
  REGION 1..17: note = 8B6 heavy chain CDR2
YINPYNDGTKYNEKFKG

SEQ ID NO: 30 - protein, 11 aa, synthetic construct
  REGION 1..11: note = 8B6 heavy chain CDR3
GYYRYGYTMDY

SEQ ID NO: 31 - protein, 11 aa, synthetic construct
  REGION 1..11: note = 8B6 light chain CDR1
RASQNFSDYLH

SEQ ID NO: 32 - protein, 7 aa, synthetic construct
  REGION 1..7: note = 8B6 light chain CDR2
YVSHSIS

SEQ ID NO: 33 - protein, 9 aa, synthetic construct
  REGION 1..9: note = 8B6 light chain CDR3
QNGHSFPPT

SEQ ID NO: 34 - protein, 107 aa, synthetic construct
  REGION 1..107: note = Humanized antibody 3-11-1
EIVLTQSPATLSLSPGERATLSCRASQSVSSYLAWYQQKPGQAPRLLIYDASNRATGIPARFSGSGSGTDFTLTISSLEPEDFAVYYCQQRSNWPWTFGQGTKVEIK

SEQ ID NO: 35 - protein, 109 aa, synthetic construct
  REGION 1..109: note = Humanized antibody 3-07-4
EVQLVESGGGLVQPGGSLRLSCAASGFTFSSYWMSWVRQAPGKGLEWVANIKQDGSEKYYVDSVKGRFTISRDNAKNSLYLQMNSLRAEDTAVYYCARWGQGTLVTVSS

SEQ ID NO: 36 - protein, 117 aa, synthetic construct
  REGION 1..117: note = Humanized antibody hu5F9-vh1
QVQLVQSGAEVKKPGASVKVSCKASGYTFTNYNMHWVRQAPGQGLEWIGTIYPGNDDTSYNQKFKDKATLTADKSTSTAYMELSSLRSEDTAVYYCARGGYRAMDYWGQGTLVTVSS

SEQ ID NO: 37 - protein, 117 aa, synthetic construct
  REGION 1..117: note = Humanized antibody hu5F9-vh2
QVQLVQSGAEVKKPGASVKVSCKASGYTFTNYNMHWVRQAPGQRLEWMGTIYPGNDDTSYNQKFKDRVTITADTSASTAYMELSSLRSEDTAVYYCARGGYRAMDYWGQGTLVTVSS

SEQ ID NO: 38 - protein, 117 aa, synthetic construct
  REGION 1..117: note = Humanized antibody hu5F9-vh3
QVQLVQSGAEVKKPGASVKVSCKASGYTFTNYNMHWVRQAPGQRLEWIGTIYPGNDDTSYNQKFKDRATLTADKSASTAYMELSSLRSEDTAVYYCARGGYRAMDYWGQGTLVTVSS

SEQ ID NO: 39 - protein, 98 aa, synthetic construct
  REGION 1..98: note = Humanized antibody IGHV1-03-01
QVQLVQSGAEVKKPGASVKVSCKASGYTFTSYAMHWVRQAPGQRLEWMGWINAGNGNTKYSQKFQGRVTITRDTSASTAYMELSSLRSEDTAVYYCAR

SEQ ID NO: 40 - protein, 98 aa, synthetic construct
  REGION 1..98: note = Humanized antibody IGHV1-46-03
QVQLVQSGAEVKKPGASVKVSCKASGYTFTSYYMHWVRQAPGQGLEWMGIINPSGGSTSYAQKFQGRVTMTRDTSTSTVYMELSSLRSEDTAVYYCAR

SEQ ID NO: 41 - protein, 112 aa, synthetic construct
  REGION 1..112: note = Humanized antibody hu5F9-vl1
DVVMTQSPLSLPVTPGEPASISCRSSQSIVYSNGNTYLGWYLQKPGQSPKLLIYKVSNRFSGVPDRFSGSGSGTDFTLKISRVEAEDVGVYHCFQGSHVPYTFGGGTKVEIK

SEQ ID NO: 42 - protein, 112 aa, synthetic construct
  REGION 1..112: note = Humanized antibody hu5F9-vl2
DIVMTQSPLSLPVTPGEPASISCRSSQSIVYSNGNTYLGWYLQKPGQSPQLLIYKVSNRFSGVPDRFSGSGSGTDFTLKISRVEAEDVGVYYCFQGSHVPYTFGQGTKLEIK

SEQ ID NO: 43 - protein, 112 aa, synthetic construct
  REGION 1..112: note = Humanized antibody hu5F9-vl3
DVVMTQSPLSLPVTPGEPASISCRSSQSIVYSNGNTYLGWYLQKPGQSPQLLIYKVSNRFSGVPDRFSGSGSGTDFTLKISRVEAEDVGVYHCFQGSHVPYTFGQGTKLEIK

SEQ ID NO: 44 - protein, 100 aa, synthetic construct
  REGION 1..100: note = Humanized antibody IGKV2-28-01
DIVMTQSPLSLPVTPGEPASISCRSSQSLLHSNGYNYLDWYLQKPGQSPQLLIYLGSNRASGVPDRFSGSGSGTDFTLKISRVEAEDVGVYYCMQALQTP

SEQ ID NO: 45 - DNA, 43 bp, synthetic construct
  misc_feature 1..43: note = Synthetic primer
  source 1..43: mol_type = other DNA
cagacccgtcgacatgaacttcgggctcagcttgattttcctt

SEQ ID NO: 46 - DNA, 45 bp, synthetic construct
  misc_feature 1..45: note = Synthetic primer
  source 1..45: mol_type = other DNA
gcccttggtgctagctgaggagacggtgactgaggttccttgacc

SEQ ID NO: 47 - DNA, 45 bp, synthetic construct
  misc_feature 1..45: note = Synthetic primer
  source 1..45: mol_type = other DNA
cgccatcacagatctatggtgtccacttctcagctccttggactt

SEQ ID NO: 48 - DNA, 45 bp, synthetic construct
  misc_feature 1..45: note = Synthetic primer
  source 1..45: mol_type = other DNA
tgcagccaccgtacgtttgatttccagcttggtgcctccaccgaa